European Patent Application EP 4 421 084 A1, published August 28, 2024. Title: Chimeric proteins and their use as an antigen detecting system. Applicant: Consejo Superior de Investigaciones Cientificas (CSIC). The sequence listing filed with the application follows.

SEQUENCE LISTING (67 sequences)

SEQ ID NO: 1 - protein, 140 aa, synthetic construct
  source 1..140: note = Antigen binding domain; note (original language) = Dominio de unión al antigeno; organism (original language) = Construccion sintetica
MAQVQLQESGGGLVQAGGSLLLSCAASGRTFSSYAMGWFRQAPGKEREFVAAINWSGGSTSYADSVKGRFTISRDNTKNTVYLQMNSLKPEDTAAFYCAATYNPYSRDHYFPRMTTEYDYWGQGTQVTVSSEPKTPKPQP

SEQ ID NO: 2 - protein, 501 aa, Escherichia coli
  source 1..501: note = beta-barrel domain from an intimin protein; note (original language) = dominio barril-beta de la proteina intimina
KSNMTDDKALNYAAQQAASLGSQLQSRSLNGDYAKDTALGIAGNQASSQLQAWLQHYGTAEVNLQSGNNFDGSSLDFLLPFYDSEKMLAFGQVGARYIDSRFTANLGAGQRFFLPANMLGYNVFIDQDFSGDNTRLGIGGEYWRDYFKSSVNGYFRMSGWHESYNKKDYDERPANGFDIRFNGYLPSYPALGAKLIYEQYYGDNVALFNSDKLQSNPGAATVGVNYTPIPLVTMGIDYRHGTGNENDLLYSMQFRYQFDKSWSQQIEPQYVNELRTLSGSRYDLVQRNNNIILEYKKQDILSLNIPHDINGTEHSTQKIQLIVKSKYGLDRIVWDDSALRSQGGQIQHSGSQSAQDYQAILPAYVQGGSNIYKVTARAYDRNGNSSNNVQLTITVLSNGQVVDQVGVTDFTADKTSAKADNADTITYTATVKKNGVAQANVPVSFNIVSGTATLGANSAKTDANGKATVTLKSSTPGQVVVSAKTAEMTSALNASAVIFFD

SEQ ID NO: 3 - protein, 451 aa, Yersinia pseudotuberculosis
  source 1..451: note = beta-barrel domain from an invasin protein; note (original language) = dominio barril-beta de la proteina invasina
KYDANAPQQVQPYSVSSSAFENLHPNNEMESSINPFSASDTERNAAIIDRANKEQETEAVNKMISTGARLAASGRASDVAHSMVGDAVNQEIKQWLNRFGTAQVNLNFDKNFSLKESSLDWLAPWYDSASFLFFSQLGIRNKDSRNTLNLGVGIRTLENGWLYGLNTFYDNDLTGHNHRIGLGAEAWTDYLQLAANGYFRLNGWHSSRDFSDYKERPATGGDLRANAYLPALPQLGGKLMYEQYTGERVALFGKDNLQRNPYAVTAGINYTPVPLLTVGVDQRMGKSSKHETQWNLQMNYRFGESFQSQLSPSAVAGTRLLAESRYNLVDRNNNIVLEYQKQQVVKLTLSPATISGLPGQVYQVNAQVQGASAVREIVWSDAELIAAGGTLTPLSTTQFNLVLPPYKRTAQVSRVTDDLTANFYSLSALAVDHQGNRSNSFTLSVTVQQPQ

SEQ ID NO: 4 - protein, 339 aa, Escherichia coli
  source 1..339: note = beta-barrel domain from an EhaA autotransporter protein; note (original language) = Dominio barril-beta de la proteina autotranspordora EhaA
TPTPGPDLNVDNDLRPEAGSYIANLAAANTMFTTRLHERLGNTYYTDMVTGEQKQTTMWMRHEGGHNKWRDGSGQLKTQSNRYVLQLGGDVAQWSQNGSDRWHVGVMAGYGNSDSKTISSRTGYRAKASVNGYSTGLYATWYADDESRNGAYLDSWAQYSWFDNTVKGDDLQSESYKSKGFTASLEAGYKHKLAEFNGSQGTRNEWYVQPQAQVTWMGVKADKHRESNGTLVHSNGDGNVQTRLGVKTWLKSHHKMDDGKSREFQPFVEVNWLHNSKDFSTSMDGVSVTQDGARNIAEIKTGVEGQLNANLNVWGNVGVQVADRGYNDTSAMVGIKWQF

SEQ ID NO: 5 - protein, 11 aa, synthetic construct
  source 1..11: note = reporter protein domain; note (original language) = dominio de proteina reportera
VTGYRLFEEIL

SEQ ID NO: 6 - protein, 158 aa, synthetic construct
  source 1..158: note = reporter protein domain; note (original language) = dominio de proteina reportera
VFTLEDFVGDWEQTAAYNLDQVLEQGGVSSLLQNLAVSVTPIQRIVRSGENALKIDIHVIIPYEGLSADQMAQIEEVFKVVYPVDDHHFKVILPYGTLVIDGVTPNMLNYFGRPYEGIAVFDGKKITVTGTLWNGNKIIDERLITPDGSMLFRVTINS

SEQ ID NO: 7 - protein, 51 aa, synthetic construct
  source 1..51: note = signal peptide; note (original language) = peptido señal
MMVFQPISEFLLIRNAGMSMYFNKIISFNIISRIVICIFLICGMFMAGASE

SEQ ID NO: 8 - protein, 43 aa, synthetic construct
  source 1..43: note = signal peptide; note (original language) = peptido señal
MITHGCYTRTRHKHKLKKTLIMLSAGLGLFFYVNQNSFANGEN

SEQ ID NO: 9 - protein, 18 aa, synthetic construct
  source 1..18: note = signal peptide; note (original language) = peptido señal
MKYLLPTAAAGLLLLAAQ

SEQ ID NO: 10 - protein, 887 aa, synthetic construct
  source 1..887: note = Chimeric protein; note (original language) = Proteina quimerica
MITHGCYTRTRHKHKLKKTLIMLSAGLGLFFYVNQNSFANGENEFGGGSVFTLEDFVGDWEQTAAYNLDQVLEQGGVSSLLQNLAVSVTPIQRIVRSGENALKIDIHVIIPYEGLSADQMAQIEEVFKVVYPVDDHHFKVILPYGTLVIDGVTPNMLNYFGRPYEGIAVFDGKKITVTGTLWNGNKIIDERLITPDGSMLFRVTINSGGGSPRKSNMTDDKALNYAAQQAASLGSQLQSRSLNGDYAKDTALGIAGNQASSQLQAWLQHYGTAEVNLQSGNNFDGSSLDFLLPFYDSEKMLAFGQVGARYIDSRFTANLGAGQRFFLPANMLGYNVFIDQDFSGDNTRLGIGGEYWRDYFKSSVNGYFRMSGWHESYNKKDYDERPANGFDIRFNGYLPSYPALGAKLIYEQYYGDNVALFNSDKLQSNPGAATVGVNYTPIPLVTMGIDYRHGTGNENDLLYSMQFRYQFDKSWSQQIEPQYVNELRTLSGSRYDLVQRNNNIILEYKKQDILSLNIPHDINGTEHSTQKIQLIVKSKYGLDRIVWDDSALRSQGGQIQHSGSQSAQDYQAILPAYVQGGSNIYKVTARAYDRNGNSSNNVQLTITVLSNGQVVDQVGVTDFTADKTSAKADNADTITYTATVKKNGVAQANVPVSFNIVSGTATLGANSAKTDANGKATVTLKSSTPGQVVVSAKTAEMTSALNASAVIFFDVDGAPVPYPDPLEPAQPAMAQVQLQESGGGLVQAGGSLLLSCAASGRTFSSYAMGWFRQAPGKEREFVAAINWSGGSTSYADSVKGRFTISRDNTKNTVYLQMNSLKPEDTAAFYCAATYNPYSRDHYFPRMTTEYDYWGQGTQVTVSSEPKTPKPQPAAAEQKLISEEDAAA

SEQ ID NO: 11 - protein, 740 aa, synthetic construct
  source 1..740: note = Chimeric protein; note (original language) = Proteina quimerica
MITHGCYTRTRHKHKLKKTLIMLSAGLGLFFYVNQNSFANGENEFGGGSVTGYRLFEEILGGGSPRKSNMTDDKALNYAAQQAASLGSQLQSRSLNGDYAKDTALGIAGNQASSQLQAWLQHYGTAEVNLQSGNNFDGSSLDFLLPFYDSEKMLAFGQVGARYIDSRFTANLGAGQRFFLPANMLGYNVFIDQDFSGDNTRLGIGGEYWRDYFKSSVNGYFRMSGWHESYNKKDYDERPANGFDIRFNGYLPSYPALGAKLIYEQYYGDNVALFNSDKLQSNPGAATVGVNYTPIPLVTMGIDYRHGTGNENDLLYSMQFRYQFDKSWSQQIEPQYVNELRTLSGSRYDLVQRNNNIILEYKKQDILSLNIPHDINGTEHSTQKIQLIVKSKYGLDRIVWDDSALRSQGGQIQHSGSQSAQDYQAILPAYVQGGSNIYKVTARAYDRNGNSSNNVQLTITVLSNGQVVDQVGVTDFTADKTSAKADNADTITYTATVKKNGVAQANVPVSFNIVSGTATLGANSAKTDANGKATVTLKSSTPGQVVVSAKTAEMTSALNASAVIFFDVDGAPVPYPDPLEPAQPAMAQVQLQESGGGLVQAGGSLLLSCAASGRTFSSYAMGWFRQAPGKEREFVAAINWSGGSTSYADSVKGRFTISRDNTKNTVYLQMNSLKPEDTAAFYCAATYNPYSRDHYFPRMTTEYDYWGQGTQVTVSSEPKTPKPQPAAAEQKLISEEDAAA

SEQ ID NO: 12 - protein, 841 aa, synthetic construct
  source 1..841: note = chimeric protein; note (original language) = proteina quimerica
MMVFQPISEFLLIRNAGMSMYFNKIISFNIISRIVICIFLICGMFMAGASEGGGSVFTLEDFVGDWEQTAAYNLDQVLEQGGVSSLLQNLAVSVTPIQRIVRSGENALKIDIHVIIPYEGLSADQMAQIEEVFKVVYPVDDHHFKVILPYGTLVIDGVTPNMLNYFGRPYEGIAVFDGKKITVTGTLWNGNKIIDERLITPDGSMLFRVTINSGGGSKYDANAPQQVQPYSVSSSAFENLHPNNEMESSINPFSASDTERNAAIIDRANKEQETEAVNKMISTGARLAASGRASDVAHSMVGDAVNQEIKQWLNRFGTAQVNLNFDKNFSLKESSLDWLAPWYDSASFLFFSQLGIRNKDSRNTLNLGVGIRTLENGWLYGLNTFYDNDLTGHNHRIGLGAEAWTDYLQLAANGYFRLNGWHSSRDFSDYKERPATGGDLRANAYLPALPQLGGKLMYEQYTGERVALFGKDNLQRNPYAVTAGINYTPVPLLTVGVDQRMGKSSKHETQWNLQMNYRFGESFQSQLSPSAVAGTRLLAESRYNLVDRNNNIVLEYQKQQVVKLTLSPATISGLPGQVYQVNAQVQGASAVREIVWSDAELIAAGGTLTPLSTTQFNLVLPPYKRTAQVSRVTDDLTANFYSLSALAVDHQGNRSNSFTLSVTVQQPQVDGAPVPYPDPLEPAQPAMAQVQLQESGGGLVQAGGSLLLSCAASGRTFSSYAMGWFRQAPGKEREFVAAINWSGGSTSYADSVKGRFTISRDNTKNTVYLQMNSLKPEDTAAFYCAATYNPYSRDHYFPRMTTEYDYWGQGTQVTVSSEPKTPKPQPAAAEQKLISEEDAAA

SEQ ID NO: 13 - protein, 694 aa, synthetic construct
  source 1..694: note = Chimeric protein; note (original language) = Proteina quimerica
MMVFQPISEFLLIRNAGMSMYFNKIISFNIISRIVICIFLICGMFMAGASEGGGSVTGYRLFEEILGGGSKYDANAPQQVQPYSVSSSAFENLHPNNEMESSINPFSASDTERNAAIIDRANKEQETEAVNKMISTGARLAASGRASDVAHSMVGDAVNQEIKQWLNRFGTAQVNLNFDKNFSLKESSLDWLAPWYDSASFLFFSQLGIRNKDSRNTLNLGVGIRTLENGWLYGLNTFYDNDLTGHNHRIGLGAEAWTDYLQLAANGYFRLNGWHSSRDFSDYKERPATGGDLRANAYLPALPQLGGKLMYEQYTGERVALFGKDNLQRNPYAVTAGINYTPVPLLTVGVDQRMGKSSKHETQWNLQMNYRFGESFQSQLSPSAVAGTRLLAESRYNLVDRNNNIVLEYQKQQVVKLTLSPATISGLPGQVYQVNAQVQGASAVREIVWSDAELIAAGGTLTPLSTTQFNLVLPPYKRTAQVSRVTDDLTANFYSLSALAVDHQGNRSNSFTLSVTVQQPQVDGAPVPYPDPLEPAQPAMAQVQLQESGGGLVQAGGSLLLSCAASGRTFSSYAMGWFRQAPGKEREFVAAINWSGGSTSYADSVKGRFTISRDNTKNTVYLQMNSLKPEDTAAFYCAATYNPYSRDHYFPRMTTEYDYWGQGTQVTVSSEPKTPKPQPAAAEQKLISEEDAAA

SEQ ID NO: 14 - protein, 714 aa, synthetic construct
  source 1..714: note = Chimeric protein; note (original language) = Proteina quimerica
MKYLLPTAAAGLLLLAAQPAMAQVQLQESGGGLVQAGGSLLLSCAASGRTFSSYAMGWFRQAPGKEREFVAAINWSGGSTSYADSVKGRFTISRDNTKNTVYLQMNSLKPEDTAAFYCAATYNPYSRDHYFPRMTTEYDYWGQGTQVTVSSEPKTPKPQPAAAAGAEFVDGAPVPYPDPLEPIDNSAAISMANPRPPTPRTPTPGPDLNVDNDLRPEAGSYIANLAAANTMFTTRLHERLGNTYYTDMVTGEQKQTTMWMRHEGGHNKWRDGSGQLKTQSNRYVLQLGGDVAQWSQNGSDRWHVGVMAGYGNSDSKTISSRTGYRAKASVNGYSTGLYATWYADDESRNGAYLDSWAQYSWFDNTVKGDDLQSESYKSKGFTASLEAGYKHKLAEFNGSQGTRNEWYVQPQAQVTWMGVKADKHRESNGTLVHSNGDGNVQTRLGVKTWLKSHHKMDDGKSREFQPFVEVNWLHNSKDFSTSMDGVSVTQDGARNIAEIKTGVEGQLNANLNVWGNVGVQVADRGYNDTSAMVGIKWQFGQGEAAPVVAPAPAPAPVFTLEDFVGDWEQTAAYNLDQVLEQGGVSSLLQNLAVSVTPIQRIVRSGENALKIDIHVIIPYEGLSADQMAQIEEVFKVVYPVDDHHFKVILPYGTLVIDGVTPNMLNYFGRPYEGIAVFDGKKITVTGTLWNGNKIIDERLITPDGSMLFRVTINS

SEQ ID NO: 15 - protein, 557 aa, synthetic construct
  source 1..557: note = Chimeric protein; note (original language) = proteina quimerica
MKYLLPTAAAGLLLLAAQPAMAQVQLQESGGGLVQAGGSLLLSCAASGRTFSSYAMGWFRQAPGKEREFVAAINWSGGSTSYADSVKGRFTISRDNTKNTVYLQMNSLKPEDTAAFYCAATYNPYSRDHYFPRMTTEYDYWGQGTQVTVSSEPKTPKPQPAAAAGAEFVDGAPVPYPDPLEPIDNSAAISMANPRPPTPRTPTPGPDLNVDNDLRPEAGSYIANLAAANTMFTTRLHERLGNTYYTDMVTGEQKQTTMWMRHEGGHNKWRDGSGQLKTQSNRYVLQLGGDVAQWSQNGSDRWHVGVMAGYGNSDSKTISSRTGYRAKASVNGYSTGLYATWYADDESRNGAYLDSWAQYSWFDNTVKGDDLQSESYKSKGFTASLEAGYKHKLAEFNGSQGTRNEWYVQPQAQVTWMGVKADKHRESNGTLVHSNGDGNVQTRLGVKTWLKSHHKMDDGKSREFQPFVEVNWLHNSKDFSTSMDGVSVTQDGARNIAEIKTGVEGQLNANLNVWGNVGVQVADRGYNDTSAMVGIKWQFGQGGGGSVTGYRLFEEIL

SEQ ID NO: 16 - DNA, 2664 bp, synthetic construct
  source 1..2664: mol_type = other DNA; note = nucleotide sequence encoding chimeric protein with SEQ ID NO: 10; note (original language) = secuencia de nucleotidos que codifica la proteina quimerica con SEQ ID NO: 10.
atgattactcatggttgttatacccggacccggcacaagcataagctaaaaaaaacattgattatgcttagtgctggtttaggattgtttttttatgttaatcagaactcatttgcaaatggtgaaaatgaattcggtgggggaagcgtcttcacactcgaagatttcgttggggactgggaacagacagccgcctacaacctggaccaagtccttgaacagggaggtgtgtccagtttgctgcaaaatctcgccgtgtccgtaactccgatccaaaggattgtccggagcggtgaaaatgccctgaagatcgacatccatgtcatcatcccgtatgaaggtctgagcgccgaccaaatggcccagatcgaagaggtgtttaaggtggtgtaccctgtggatgatcatcactttaaggtgatcctgccctatggcacactggtaatcgacggggttacgccgaacatgctgaactatttcggacggccgtatgaaggcatcgccgtgttcgacggcaaaaagatcactgtaacagggaccctgtggaacggcaacaaaattatcgacgagcgcctgatcacccccgacggctccatgctgttccgagtaaccatcaacagcggcggagggtctccgcggaaaagcaacatgaccgatgacaaggcattaaattatgcggcacaacaggcggcgagtctcggtagccagcttcagtcgcgatctctgaacggcgattacgcgaaagataccgctcttggtatcgctggtaaccaggcttcgtcacagttgcaggcctggttacaacattatggaacggcagaggttaatctgcaaagtggtaataactttgacggtagttcactggacttcttattaccgttctatgattccgaaaaaatgctggcatttggtcaggtcggagcgcgttacattgactcccgctttacggcaaatttaggtgcgggtcagcgttttttccttcctgcaaacatgttgggctataacgtcttcattgatcaggatttttctggtgataatacccgtttaggtattggtggcgaatactggcgagactatttcaaaagtagcgttaacggctatttccgcatgagcggctggcatgagtcatacaataagaaagactatgatgagcgcccagcaaatggcttcgatatccgttttaatggctatctaccgtcatatccggcattaggcgccaagctgatatatgagcagtattatggtgataatgttgctttgtttaattctgataagctgcaatcgaatcctggtgcggcgaccgttggtgtaaactatactccgattcctctggtgacgatggggattgattaccgtcatggtacgggtaatgaaaatgatctcctttactcaatgcagttccgttatcagtttgataaatcgtggagccagcaaattgaaccacagtatgttaacgagttaagaacattatcaggcagccgttacgatctggttcagcgtaataacaatattattctggagtacaagaagcaggatattctttctctgaatattccgcatgatattaatggtactgaacacagtacgcagaagattcagttgatcgttaagagcaaatacggtctggatcgtatcgtctgggatgatagtgcattacgcagtcagggcggtcagattcagcatagcggaagccaaagcgcacaagactaccaggctattttgcctgcttatgtgcaaggtggcagcaatatttataaagtgacggctcgcgcctatgaccgtaatggcaatagctctaacaatgtacagcttactattaccgttctgtcgaatggtcaagttgttgaccaggttggggtaacggactttacggcggataagacttcggctaaagcggataacgccgataccattacttataccgcgacggtgaaaaagaatggggtagctcaggctaatgtccctgtttcatttaatattgtttcaggaactgcaactcttggggcaaatagtgccaaaacggatgctaacggtaaggcaaccgtaacgttgaagtcgagtacgccaggacaggtcgtcgtgtctgctaaaaccgccgagatgacttcagcacttaatgccagtgcggttatattttttgatgtcgacggtgcgccggtgccgtatccggacccgctggaaccggcccagccggccatggcccaggtgcagctgcaggagtctgggggaggattggtgcaggctgggggttctctgttgctctcctgtgcagcctctggacgcaccttcagtagctatgccatgggctggttccgccaggctccagggaaggagcgtgagtttgtagcagctattaactggagtggtggtagcacaagctatgcagactccgtgaagggccgattcacaatctccagagacaacaccaagaacacggtgtatctgcaaatgaacagcctgaaacctgaggacacggccgctttttactgtgcagctacgtacaatccatactcgcgtgatcattacttcccgcgcatgaccactgagtatgactactggggccaggggacccaggtcaccgtctcctcagaacccaagacaccaaaaccacaaccagcggccgccgaacaaaaactcatctcagaagaggatgcagctgcataa

SEQ ID NO: 17 - DNA, 2223 bp, synthetic construct
  source 1..2223: mol_type = other DNA; note = nucleotide sequence encoding the chimeric protein with SEQ ID NO: 11; note (original language) = Secuencia de nucleotidos que codifica la proteina quimerica con SEQ ID NO: 11
atgattactcatggttgttatacccggacccggcacaagcataagctaaaaaaaacattgattatgcttagtgctggtttaggattgtttttttatgttaatcagaactcatttgcaaatggtgaaaatgaattcggtgggggaagcgtgaccggctaccggctgttcgaggagattctgggcggagggtctccgcggaaaagcaacatgaccgatgacaaggcattaaattatgcggcacaacaggcggcgagtctcggtagccagcttcagtcgcgatctctgaacggcgattacgcgaaagataccgctcttggtatcgctggtaaccaggcttcgtcacagttgcaggcctggttacaacattatggaacggcagaggttaatctgcaaagtggtaataactttgacggtagttcactggacttcttattaccgttctatgattccgaaaaaatgctggcatttggtcaggtcggagcgcgttacattgactcccgctttacggcaaatttaggtgcgggtcagcgttttttccttcctgcaaacatgttgggctataacgtcttcattgatcaggatttttctggtgataatacccgtttaggtattggtggcgaatactggcgagactatttcaaaagtagcgttaacggctatttccgcatgagcggctggcatgagtcatacaataagaaagactatgatgagcgcccagcaaatggcttcgatatccgttttaatggctatctaccgtcatatccggcattaggcgccaagctgatatatgagcagtattatggtgataatgttgctttgtttaattctgataagctgcaatcgaatcctggtgcggcgaccgttggtgtaaactatactccgattcctctggtgacgatggggattgattaccgtcatggtacgggtaatgaaaatgatctcctttactcaatgcagttccgttatcagtttgataaatcgtggagccagcaaattgaaccacagtatgttaacgagttaagaacattatcaggcagccgttacgatctggttcagcgtaataacaatattattctggagtacaagaagcaggatattctttctctgaatattccgcatgatattaatggtactgaacacagtacgcagaagattcagttgatcgttaagagcaaatacggtctggatcgtatcgtctgggatgatagtgcattacgcagtcagggcggtcagattcagcatagcggaagccaaagcgcacaagactaccaggctattttgcctgcttatgtgcaaggtggcagcaatatttataaagtgacggctcgcgcctatgaccgtaatggcaatagctctaacaatgtacagcttactattaccgttctgtcgaatggtcaagttgttgaccaggttggggtaacggactttacggcggataagacttcggctaaagcggataacgccgataccattacttataccgcgacggtgaaaaagaatggggtagctcaggctaatgtccctgtttcatttaatattgtttcaggaactgcaactcttggggcaaatagtgccaaaacggatgctaacggtaaggcaaccgtaacgttgaagtcgagtacgccaggacaggtcgtcgtgtctgctaaaaccgccgagatgacttcagcacttaatgccagtgcggttatattttttgatgtcgacggtgcgccggtgccgtatccggacccgctggaaccggcccagccggccatggcccaggtgcagctgcaggagtctgggggaggattggtgcaggctgggggttctctgttgctctcctgtgcagcctctggacgcaccttcagtagctatgccatgggctggttccgccaggctccagggaaggagcgtgagtttgtagcagctattaactggagtggtggtagcacaagctatgcagactccgtgaagggccgattcacaatctccagagacaacaccaagaacacggtgtatctgcaaatgaacagcctgaaacctgaggacacggccgctttttactgtgcagctacgtacaatccatactcgcgtgatcattacttcccgcgcatgaccactgagtatgactactggggccaggggacccaggtcaccgtctcctcagaacccaagacaccaaaaccacaaccagcggccgccgaacaaaaactcatctcagaagaggatgcagctgcataa

SEQ ID NO: 18 - DNA, 2526 bp, synthetic construct
  source 1..2526: mol_type = other DNA; note = nucleotide sequence encoding chimeric protein with SEQ ID NO: 12; note (original language) = secuencia de nucleotidos que codifica la proteina quimerica con SEQ ID NO: 12
atgatggttttccagccaatcagtgagtttctcttgataaggaatgcgggaatgtctatgtattttaataaaataatttcatttaatattatttcacgaatagttatttgtatctttttgatatgtggaatgttcatggctggggcttcagaaggtgggggaagcgtcttcacactcgaagatttcgttggggactgggaacagacagccgcctacaacctggaccaagtccttgaacagggaggtgtgtccagtttgctgcaaaatctcgccgtgtccgtaactccgatccaaaggattgtccggagcggtgaaaatgccctgaagatcgacatccatgtcatcatcccgtatgaaggtctgagcgccgaccaaatggcccagatcgaagaggtgtttaaggtggtgtaccctgtggatgatcatcactttaaggtgatcctgccctatggcacactggtaatcgacggggttacgccgaacatgctgaactatttcggacggccgtatgaaggcatcgccgtgttcgacggcaaaaagatcactgtaacagggaccctgtggaacggcaacaaaattatcgacgagcgcctgatcacccccgacggctccatgctgttccgagtaaccatcaacagcggcggagggtctaaatatgatgctaacgcaccgcaacaggtccagccttattctgtctcttcatctgcatttgaaaatctccatcctaataatgaaatggagagttcaatcaatcccttttccgcatcggatacagaaagaaatgctgcaataatagatcgcgccaataaggagcaggagactgaagcggtgaataagatgataagcaccggggccaggttagctgcatcaggcagggcatctgatgttgctcactcaatggtgggcgatgcggttaatcaagaaatcaaacagtggttaaatcgattcggtacggctcaagttaatctgaattttgacaaaaatttttcgctaaaagaaagctctcttgattggctggctccttggtatgactctgcttcattcctcttttttagtcagttaggtattcgcaataaagacagccgcaacacacttaaccttggcgtcgggatacgtacattggagaacggttggctgtacggacttaatactttttatgataatgatttgaccggccacaaccaccgtatcggtcttggtgccgaggcctggaccgattatttacagttggctgccaatgggtattttcgcctcaatggatggcactcgtcgcgtgatttctccgactataaagagcgcccagccactgggggggatttgcgcgcgaatgcttatttacctgcactcccacaactgggggggaagttgatgtatgagcaatacaccggtgagcgtgttgctttatttggtaaagataatctgcaacgcaacccttatgccgtgactgccgggatcaattacacccccgtgcctctactcactgtcggggtagatcagcgtatggggaaaagcagtaagcatgaaacacagtggaacctccaaatgaactatcgctttggcgagagttttcagtcgcaacttagcccttcagcggtggcaggaacacgtctactggcggagagccgctataaccttgtcgatcgtaacaataatatcgtgttggagtatcagaaacagcaggtggttaaactgacattatcgccagcaactatctccggcctgccgggtcaggtttatcaggtgaacgcacaagtacaaggggcatctgctgtaagggaaattgtctggagtgatgccgaactgattgccgctggcggcacattaacaccactgagtaccacacaattcaacttggttttaccgccttataaacgcacagcacaagtgagtcgggtaacggacgacctgacagccaacttttattcgcttagtgcgctcgcggttgatcaccaaggaaaccgatctaactcattcacattgagcgtcaccgttcagcagcctcaggtcgacggtgcgccggtgccgtatccggacccgctggaaccggcccagccggccatggcccaggtgcagctgcaggagtctgggggaggattggtgcaggctgggggttctctgttgctctcctgtgcagcctctggacgcaccttcagtagctatgccatgggctggttccgccaggctccagggaaggagcgtgagtttgtagcagctattaactggagtggtggtagcacaagctatgcagactccgtgaagggccgattcacaatctccagagacaacaccaagaacacggtgtatctgcaaatgaacagcctgaaacctgaggacacggccgctttttactgtgcagctacgtacaatccatactcgcgtgatcattacttcccgcgcatgaccactgagtatgactactggggccaggggacccaggtcaccgtctcctcagaacccaagacaccaaaaccacaaccagcggccgccgaacaaaaactcatctcagaagaggatgcagctgcataa

SEQ ID NO: 19 - DNA, 2085 bp, synthetic construct
  source 1..2085: mol_type = other DNA; note = Nucleotide sequence encoding chimeric protein with SEQ ID NO: 13; note (original language) = secuencia de nucleotidos que codifica la proteina quimerica SEQ ID NO: 13
atgatggttttccagccaatcagtgagtttctcttgataaggaatgcgggaatgtctatgtattttaataaaataatttcatttaatattatttcacgaatagttatttgtatctttttgatatgtggaatgttcatggctggggcttcagaaggtgggggaagcgtgaccggctaccggctgttcgaggagattctgggcggagggtctaaatatgatgctaacgcaccgcaacaggtccagccttattctgtctcttcatctgcatttgaaaatctccatcctaataatgaaatggagagttcaatcaatcccttttccgcatcggatacagaaagaaatgctgcaataatagatcgcgccaataaggagcaggagactgaagcggtgaataagatgataagcaccggggccaggttagctgcatcaggcagggcatctgatgttgctcactcaatggtgggcgatgcggttaatcaagaaatcaaacagtggttaaatcgattcggtacggctcaagttaatctgaattttgacaaaaatttttcgctaaaagaaagctctcttgattggctggctccttggtatgactctgcttcattcctcttttttagtcagttaggtattcgcaataaagacagccgcaacacacttaaccttggcgtcgggatacgtacattggagaacggttggctgtacggacttaatactttttatgataatgatttgaccggccacaaccaccgtatcggtcttggtgccgaggcctggaccgattatttacagttggctgccaatgggtattttcgcctcaatggatggcactcgtcgcgtgatttctccgactataaagagcgcccagccactgggggggatttgcgcgcgaatgcttatttacctgcactcccacaactgggggggaagttgatgtatgagcaatacaccggtgagcgtgttgctttatttggtaaagataatctgcaacgcaacccttatgccgtgactgccgggatcaattacacccccgtgcctctactcactgtcggggtagatcagcgtatggggaaaagcagtaagcatgaaacacagtggaacctccaaatgaactatcgctttggcgagagttttcagtcgcaacttagcccttcagcggtggcaggaacacgtctactggcggagagccgctataaccttgtcgatcgtaacaataatatcgtgttggagtatcagaaacagcaggtggttaaactgacattatcgccagcaactatctccggcctgccgggtcaggtttatcaggtgaacgcacaagtacaaggggcatctgctgtaagggaaattgtctggagtgatgccgaactgattgccgctggcggcacattaacaccactgagtaccacacaattcaacttggttttaccgccttataaacgcacagcacaagtgagtcgggtaacggacgacctgacagccaacttttattcgcttagtgcgctcgcggttgatcaccaaggaaaccgatctaactcattcacattgagcgtcaccgttcagcagcctcaggtcgacggtgcgccggtgccgtatccggacccgctggaaccggcccagccggccatggcccaggtgcagctgcaggagtctgggggaggattggtgcaggctgggggttctctgttgctctcctgtgcagcctctggacgcaccttcagtagctatgccatgggctggttccgccaggctccagggaaggagcgtgagtttgtagcagctattaactggagtggtggtagcacaagctatgcagactccgtgaagggccgattcacaatctccagagacaacaccaagaacacggtgtatctgcaaatgaacagcctgaaacctgaggacacggccgctttttactgtgcagctacgtacaatccatactcgcgtgatcattacttcccgcgcatgaccactgagtatgactactggggccaggggacccaggtcaccgtctcctcagaacccaagacaccaaaaccacaaccagcggccgccgaacaaaaactcatctcagaagaggatgcagctgcataa

SEQ ID NO: 20 - DNA, 2145 bp, synthetic construct
  source 1..2145: mol_type = other DNA; note = nucleotide sequence encoding chimeric protein with SEQ ID NO: 14; note (original language) = secuencia de nucleotidos que codifica la proteina quimerica con SEQ ID NO: 14
atgaaatacctattgcctacggcagccgctggattgttattactcgcggcccagccggccatggcccaggtgcagctgcaggagtctgggggaggattggtgcaggctgggggttctctgttgctctcctgtgcagcctctggacgcaccttcagtagctatgccatgggctggttccgccaggctccagggaaggagcgtgagtttgtagcagctattaactggagtggtggtagcacaagctatgcagactccgtgaagggccgattcacaatctccagagacaacaccaagaacacggtgtatctgcaaatgaacagcctgaaacctgaggacacggccgctttttactgtgcagctacgtacaatccatactcgcgtgatcattacttcccgcgcatgaccactgagtatgactactggggccaggggacccaggtcaccgtctcctcagaacccaagacaccaaaaccacaaccagcggccgctgcgggggccgaattcgtcgacggtgcgccggtgccgtatccggatccgctggaaccgatcgacaattcagccgcaattagtatggcaaatccacgtccaccaacaccgcggacacctacgccgggtccggatctgaatgtggataatgacctgcgaccggaggcgggtagctacattgcgaaccttgcagcagcgaataccatgttcaccacgcgtctgcatgagcgtctgggtaatacgtactataccgacatggtgacgggtgagcagaaacaaaccactatgtggatgcgccatgaaggtggtcataataaatggcgtgatggcagcggccagctgaaaacccaaagcaatcgctatgttctgcaactgggaggcgatgtcgcgcagtggagccaaaacggcagcgaccgctggcatgttggggtcatggcgggatatggcaacagcgacagcaaaaccatttcctcgcgaaccggttatcgtgcaaaagcgagtgtgaacggatatagcacaggcctctatgccacctggtatgccgatgacgagtcgcgtaatggcgcgtatctcgacagttgggcgcagtacagctggtttgataacacagtgaaaggggatgacttacaaagtgaatcctataaatcaaaaggatttaccgcttcactggaagctggatacaaacacaaattagctgaatttaatggcagccagggaacgcgtaatgaatggtatgttcagccgcaagcacaggttacctggatgggagtcaaagccgataagcaccgcgaaagcaacggaaccctcgttcatagcaacggtgatggcaatgttcaaacccgacttggcgtaaaaacctggctgaagagccaccataaaatggatgacggtaaatcccgcgagttccagccgtttgtagaagtgaactggctacataacagtaaggatttcagcaccagtatggatggcgtgtctgtcactcaggatggagcccgaaatattgctgagataaaaaccggggtggaaggacagctaaatgccaacctgaatgtctgggggaatgtgggcgttcaggttgccgataggggatataatgacacctctgcaatggttggcattaagtggcaattcggtcaaggagaagcagcacctgtggttgcgcctgcaccggctcctgcaccagtcttcacactcgaagatttcgttggggactgggaacagacagccgcctacaacctggaccaagtccttgaacagggaggtgtgtccagtttgctgcaaaatctcgccgtgtccgtaactccgatccaaaggattgtccggagcggtgaaaatgccctgaagatcgacatccatgtcatcatcccgtatgaaggtctgagcgccgaccaaatggcccagatcgaagaggtgtttaaggtggtgtaccctgtggatgatcatcactttaaggtgatcctgccctatggcacactggtaatcgacggggttacgccgaacatgctgaactatttcggacggccgtatgaaggcatcgccgtgttcgacggcaaaaagatcactgtaacagggaccctgtggaacggcaacaaaattatcgacgagcgcctgatcacccccgacggctccatgctgttccgagtaaccatcaacagctaa

SEQ ID NO: 21 - DNA, 1674 bp, synthetic construct
  source 1..1674: mol_type = other DNA; note = nucleotide sequence encoding chimeric protein with SEQ ID NO: 15; note (original language) = secuencia de nucleotidos que codifica la proteina quimerica SEQ ID NO: 15
atgaaatacctattgcctacggcagccgctggattgttattactcgcggcccagccggccatggcccaggtgcagctgcaggagtctgggggaggattggtgcaggctgggggttctctgttgctctcctgtgcagcctctggacgcaccttcagtagctatgccatgggctggttccgccaggctccagggaaggagcgtgagtttgtagcagctattaactggagtggtggtagcacaagctatgcagactccgtgaagggccgattcacaatctccagagacaacaccaagaacacggtgtatctgcaaatgaacagcctgaaacctgaggacacggccgctttttactgtgcagctacgtacaatccatactcgcgtgatcattacttcccgcgcatgaccactgagtatgactactggggccaggggacccaggtcaccgtctcctcagaacccaagacaccaaaaccacaaccagcggccgctgcgggggccgaattcgtcgacggtgcgccggtgccgtatccggatccgctggaaccgatcgacaattcagccgcaattagtatggcaaatccacgtccaccaacaccgcggacacctacgccgggtccggatctgaatgtggataatgacctgcgaccggaggcgggtagctacattgcgaaccttgcagcagcgaataccatgttcaccacgcgtctgcatgagcgtctgggtaatacgtactataccgacatggtgacgggtgagcagaaacaaaccactatgtggatgcgccatgaaggtggtcataataaatggcgtgatggcagcggccagctgaaaacccaaagcaatcgctatgttctgcaactgggaggcgatgtcgcgcagtggagccaaaacggcagcgaccgctggcatgttggggtcatggcgggatatggcaacagcgacagcaaaaccatttcctcgcgaaccggttatcgtgcaaaagcgagtgtgaacggatatagcacaggcctctatgccacctggtatgccgatgacgagtcgcgtaatggcgcgtatctcgacagttgggcgcagtacagctggtttgataacacagtgaaaggggatgacttacaaagtgaatcctataaatcaaaaggatttaccgcttcactggaagctggatacaaacacaaattagctgaatttaatggcagccagggaacgcgtaatgaatggtatgttcagccgcaagcacaggttacctggatgggagtcaaagccgataagcaccgcgaaagcaacggaaccctcgttcatagcaacggtgatggcaatgttcaaacccgacttggcgtaaaaacctggctgaagagccaccataaaatggatgacggtaaatcccgcgagttccagccgtttgtagaagtgaactggctacataacagtaaggatttcagcaccagtatggatggcgtgtctgtcactcaggatggagcccgaaatattgctgagataaaaaccggggtggaaggacagctaaatgccaacctgaatgtctgggggaatgtgggcgttcaggttgccgataggggatataatgacacctctgcaatggttggcattaagtggcaattcggacagggcggtgggggaagcgtgaccggctaccggctgttcgaggagattctgtaa

SEQ ID NO: 22 - DNA, 26 bp, synthetic construct
  source 1..26: mol_type = other DNA
catttttcacttcacaggtcaagctt

SEQ ID NO: 23 - DNA, 22 bp, synthetic construct
  source 1..22: mol_type = other DNA
ccgattcattaatgcagctggc

SEQ ID NO: 24 - DNA, 27 bp, synthetic construct
  source 1..27: mol_type = other DNA
ggtaataagaagtccagtgaactaccg

SEQ ID NO: 25 - DNA, 31 bp, synthetic construct
  source 1..31: mol_type = other DNA
ccgcggttacaacattatggaacggcagagg

SEQ ID NO: 26 - DNA, 66 bp, synthetic construct
  source 1..66: mol_type = other DNA
aattcggtgggggaagcgtgaccggctaccggctgttcgaggagattctgggcggagggtctccgc

SEQ ID NO: 27 - DNA, 60 bp, synthetic construct
  source 1..60: mol_type = other DNA
ggagaccctccgcccagaatctcctcgaacagccggtagccggtcacgcttcccccaccg

SEQ ID NO: 28 - DNA, 20 bp, synthetic construct
  source 1..20: mol_type = other DNA
actcggaacagcatggagcc

SEQ ID NO: 29 - DNA, 63 bp, synthetic construct
  source 1..63: mol_type = other DNA
gcgcatattgtgatggttgatgcctataaaccgaccaagggcggagggtctccgcggaaaagc

SEQ ID NO: 30 - DNA, 66 bp, synthetic construct
  source 1..66: mol_type = other DNA
cttggtcggtttataggcatcaaccatcacaatatgcgcgcttcccccaccgaattcattttcacc

SEQ ID NO: 31 - DNA, 60 bp, synthetic construct
  source 1..60: mol_type = other DNA
aaactgggcgatattgaatttatcaaggtgaacaaaggcggagggtctccgcggaaaagc

SEQ ID NO: 32 - DNA, 63 bp, synthetic construct
  source 1..63: mol_type = other DNA
tttgttcaccttgataaattcaatatcgcccagtttgcttcccccaccgaattcattttcacc

SEQ ID NO: 33 - DNA, 24 bp, synthetic construct
  source 1..24: mol_type = other DNA
catagtggtttgtttctgctcacc

SEQ ID NO: 34 - DNA, 24 bp, synthetic construct
  source 1..24: mol_type = other DNA
gggtagctacattgcgaaccttgc

SEQ ID NO: 35 - DNA, 43 bp, synthetic construct
  source 1..43: mol_type = other DNA
gcttcccccaccgccctgtccgaattgccacttaatgccaacc

SEQ ID NO: 36 - DNA, 66 bp, synthetic construct
  source 1..66: mol_type = other DNA
ggtcaagcttttacagaatctcctcgaacagccggtagccggtcacgcttcccccaccgccctgtc

SEQ ID NO: 37 - DNA, 48 bp, synthetic construct
  source 1..48: mol_type = other DNA
cggacagggcggtgggggaagcgtcttcacactcgaagatttcgttgg

SEQ ID NO: 38 - DNA, 35 bp, synthetic construct
  source 1..35: mol_type = other DNA
caagcttttagctgttgatggttactcggaacagc

SEQ ID NO: 39 - DNA, 65 bp, synthetic construct
  source 1..65: mol_type = other DNA
acctgtggttgcgcctgcaccggctcctgcaccataaaagcttgacctgtgaagtgaaaaatggc

SEQ ID NO: 40 - DNA, 60 bp, synthetic construct
  source 1..60: mol_type = other DNA
agccggtgcaggcgcaaccacaggtgctgcttctccttgaccgaattgccacttaatgcc

SEQ ID NO: 41 - DNA, 60 bp, synthetic construct
  source 1..60: mol_type = other DNA
acctgtggttgcgcctgcaccggctcctgcaccagtcttcacactcgaagatttcgttgg

SEQ ID NO: 42 - DNA, 40 bp, synthetic construct
  source 1..40: mol_type = other DNA
cacgtccaccaacaccgcgggtccccctgtatgcctccat

SEQ ID NO: 43 - DNA, 40 bp, synthetic construct
  source 1..40: mol_type = other DNA
atggaggcatacagggggacccgcggtgttggtggacgtg

SEQ ID NO: 44 - DNA, 40 bp, synthetic construct
  source 1..40: mol_type = other DNA
cacgtccaccaacaccgcggacgaatgtcactctcgcctc

SEQ ID NO: 45 - DNA, 40 bp, synthetic construct
  source 1..40: mol_type = other DNA
gaggcgagagtgacattcgtccgcggtgttggtggacgtg

SEQ ID NO: 46 - DNA, 44 bp, synthetic construct
  source 1..44: mol_type = other DNA
cacttcacaggtcaagcttttagaaggtcacattcagtgtggcc

SEQ ID NO: 47 - DNA, 44 bp, synthetic construct
  source 1..44: mol_type = other DNA
ggccacactgaatgtgaccttctaaaagcttgacctgtgaagtg

SEQ ID NO: 48 - DNA, 41 bp, synthetic construct
  source 1..41: mol_type = other DNA
ccacactgaatgtgaccttcggtcaaggagaagcagcacct

SEQ ID NO: 49 - DNA, 40 bp, synthetic construct
  source 1..40: mol_type = other DNA
ggtgctgcttctccttgaccgaaggtcacattcagtgtgg

SEQ ID NO: 50 - DNA, 40 bp, synthetic construct
  source 1..40: mol_type = other DNA
ctgcaccggctcctgcaccagtgaccggctaccggctgtt

SEQ ID NO: 51 - DNA, 40 bp, synthetic construct
  source 1..40: mol_type = other DNA
aacagccggtagccggtcactggtgcaggagccggtgcag

SEQ ID NO: 52 - DNA, 38 bp, synthetic construct
  source 1..38: mol_type = other DNA
atcgtcgaccttaacaaagtgggtatcaacactttgcc

SEQ ID NO: 53 - DNA, 22 bp, synthetic construct
  source 1..22: mol_type = other DNA
tttcttgattaaccgcatcgcc

SEQ ID NO: 54 - DNA, 25 bp, synthetic construct
  source 1..25: mol_type = other DNA
aaatgaactatcgctttggcgagag

SEQ ID NO: 55 - DNA, 24 bp, synthetic construct
  source 1..24: mol_type = other DNA
tcgccaaagcgatagttcatttgg

SEQ ID NO: 56 - DNA, 26 bp, synthetic construct
  source 1..26: mol_type = other DNA
actggtcgacctgaggctgctgaacg

SEQ ID NO: 57 - DNA, 72 bp, synthetic construct
  source 1..72: mol_type = other DNA
gtgaccggctaccggctgttcgaggagattctgggcggagggtctaaatatgatgctaacgcaccgcaacag

SEQ ID NO: 58 - DNA, 67 bp, synthetic construct
  source 1..67: mol_type = other DNA
cagaatctcctcgaacagccggtagccggtcacgcttcccccaccttctgaagccccagccatgaac

SEQ ID NO: 59 - DNA, 40 bp, synthetic construct
  source 1..40: mol_type = other DNA
tcatggctggggcttcagaaggtgggggaagcgtcttcac

SEQ ID NO: 60 - DNA, 42 bp, synthetic construct
  source 1..42: mol_type = other DNA
gtgaagacgcttcccccaccttctgaagccccagccatgaac

SEQ ID NO: 61 - DNA, 47 bp, synthetic construct
  source 1..47: mol_type = other DNA
tcaacagcggcggagggtctaaatatgatgctaacgcaccgcaacag

SEQ ID NO: 62 - DNA, 40 bp, synthetic construct
  source 1..40: mol_type = other DNA
ggtgcgttagcatcatatttagaccctccgccgctgttga

SEQ ID NO: 63 - DNA, 78 bp, synthetic construct
  source 1..78: mol_type = other DNA
gcgcatattgtgatggttgatgcctataaaccgaccaagggcggagggtctaaatatgatgctaacgcaccgcaacag

SEQ ID NO: 64 - DNA, 73 bp, synthetic construct
  source 1..73: mol_type = other DNA
cttggtcggtttataggcatcaaccatcacaatatgcgcgcttcccccaccttctgaagccccagccatgaac

SEQ ID NO: 65 - DNA, 75 bp, synthetic construct
  source 1..75: mol_type = other DNA
aaactgggcgatattgaatttatcaaggtgaacaaaggcggagggtctaaatatgatgctaacgcaccgcaacag

SEQ ID NO: 66 - DNA, 70 bp, synthetic construct
  source 1..70: mol_type = other DNA
tttgttcaccttgataaattcaatatcgcccagtttgcttcccccaccttctgaagccccagccatgaac

SEQ ID NO: 67 - protein, 17 aa, synthetic construct
GQGEAAPVVAPAPAPAP